European Patent Application EP 4 141 448 A1, published March 1, 2023. Title: PROTEIN SIGNATURES FOR DISTINGUISHING BETWEEN BACTERIAL AND VIRAL INFECTIONS. Applicant: MeMed Diagnostics Ltd. The sequence listing filed with the application follows.

SEQUENCE LISTING (24 sequences)

SEQ ID NO: 1 - protein, 224 aa, homo sapiens
MEKLLCFLVLTSLSHAFGQTDMSRKAFVFPKESDTSYVSLKAPLTKPLKAFTVCLHFYTELSSTRGYSIFSYATKRQDNEILIFWSKDIGYSFTVGGSEILFEVPEVTVAPVHICTSWESASGIVEFWVDGKPRVRKSLKKGYTVGAEASIILGQEQDSFGGNFEGSQSLVGDIGNVNMWDFVLSPDEINTIYLGGPFSPNVLNWRALKYEVQGEVFTKPQLWP

SEQ ID NO: 2 - DNA, 1805 bp, homo sapiens
acagaacccagaaaaacaactcattcgctttcatttcctcactgactataaaagaatagagaaggaagggcttcagtgaccggctgcctggctgacttacagcagtcagactctgacaggatcatggctatgatggaggtccaggggggacccagcctgggacagacctgcgtgctgatcgtgatcttcacagtgctcctgcagtctctctgtgtggctgtaacttacgtgtactttaccaacgagctgaagcagatgcaggacaagtactccaaaagtggcattgcttgtttcttaaaagaagatgacagttattgggaccccaatgacgaagagagtatgaacagcccctgctggcaagtcaagtggcaactccgtcagctcgttagaaagactccaagaatgaaaaggctctgggccgcaaaataaactcctgggaatcatcaaggagtgggcattcattcctgagcaacttgcacttgaggaatggtgaactggtcatccatgaaaaagggttttactacatctattcccaaacatactttcgatttcaggaggaaataaaagaaaacacaaagaacgacaaacaaatggtccaatatatttacaaatacacaagttatcctgaccctatattgttgatgaaaagtgctagaaatagttgttggtctaaagatgcagaatatggactctattccatctatcaagggggaatatttgagcttaaggaaaatgacagaatttttgtttctgtaacaaatgagcacttgatagacatggaccatgaagccagtttttttggggcctttttagttggctaactgacctggaaagaaaaagcaataacctcaaagtgactattcagttttcaggatgatacactatgaagatgtttcaaaaaatctgaccaaaacaaacaaacagaaaacagaaaacaaaaaaacctctatgcaatctgagtagagcagccacaaccaaaaaattctacaacacacactgttctgaaagtgactcacttatcccaagagaatgaaattgctgaaagatctttcaggactctacctcatatcagtttgctagcagaaatctagaagactgtcagcttccaaacattaatgcaatggttaacatcttctgtctttataatctactccttgtaaagactgtagaagaaagagcaacaatccatctctcaagtagtgtatcacagtagtagcctccaggtttccttaagggacaacatccttaagtcaaaagagagaagaggcaccactaaaagatcgcagtttgcctggtgcagtggctcacacctgtaatcccaacattttgggaacccaaggtgggtagatcacgagatcaagagatcaagaccatagtgaccaacatagtgaaaccccatctctactgaaagtacaaaaattagctgggtgtgttggcacatgcctgtagtcccagctacttgagaggctgaggcaagagaattgtttgaacccgggaggcagaggttgcagtgtggtgagatcatgccactacactccagcctggcgacagagcgagacttggtttcaaaaaaaaaaaaaaaaaaaacttcagtaagtacgtgttatttttttcaataaaattctattacagtatgtcatgtttgctgtagtgctcatatttattgttgtttttgttttagtactcacttgtttcataatatcaagattactaaaaatgggggaaaagacttctaatctttttttcataatatctttgacacatattacagaagaaataaatttcttacttttaatttaatatga

SEQ ID NO: 3 - DNA, 1334 bp, homo sapiens
atttcctcactgactataaaagaatagagaaggaagggcttcagtgaccggctgcctggctgacttacagcagtcagactctgacaggatcatggctatgatggaggtccaggggggacccagcctgggacagacctgcgtgctgatcgtgatcttcacagtgctcctgcagtctctctgtgtggctgtaacttacgtgtactttaccaacgagctgaagcagtttgcagaaaatgattgccagagactaatgtctgggcagcagacagggtcattgctgccatcttgaagtctaccttgctgagtctaccctgctgacctcaagccccatcaaggactggttgaccctggcctagacaaccaccgtgtttgtaacagcaccaagagcagtcaccatggaaatccacttttcagaaccaagggcttctggagctgaagaacaggcacccagtgcaagagctttcttttcagaggcacgcaaatgaaaataatccccacacgctaccttctgcccccaatgcccaagtgtggttagttagagaatatagcctcagcctatgatatgctgcaggaaactcatattttgaagtggaaaggatgggaggaggcgggggagacgtatcgtattaattatcattcttggaataaccacagcacctcacgtcaacccgccatgtgtctagtcaccagcattggccaagttctataggagaaactaccaaaattcatgatgcaagaaacatgtgagggtggagagagtgactggggcttcctctctggatttctattgttcagaaatcaatatttatgcataaaaaggtctagaaagagaaacaccaaaatgacaatgtgatctctagatggtatgattatgggtactttttttcctttttatttttctatattttacaaattttctacagggaatgttataaaaatatccatgctatccatgtataattttcatacagatttaaagaacacagcatttttatatagtcttatgagaaaacaaccatactcaaaattatgcacacacacagtctgatctcacccctgtaaacaagagatatcatccaaaggttaagtaggaggtgagaatatagctgctattagtggttgttttgttttgtttttgtgatttacttatttagtttttggagggttttttttttcttttagaaaagtgttctttacttttccatgcttccctgcttgcctgtgtatcctgaatgtatccaggctttataaactcctgggtaataatgtagctacattaacttgttaacctcccatccacttatacccaggaccttactcaattttccaggttc

SEQ ID NO: 4 - protein, 281 aa, homo sapiens [sequence omitted]

SEQ ID NO: 5 - protein, 101 aa, homo sapiens
MAMMEVQGGPSLGQTCVLIVIFTVLLQSLCVAVTYVYFTNELKQMQDKYSKSGIACFLKEDDSYWDPNDEESMNSPCWQVKWQLRQLVRKTPRMKRLWAAK

SEQ ID NO: 6 - protein, 65 aa, homo sapiens
MAMMEVQGGPSLGQTCVLIVIFTVLLQSLCVAVTYVYFTNELKQFAENDCQRLMSGQQTGSLLPS

SEQ ID NO: 7 - protein, 223 aa, homo sapiens
QDHGYDGGPGGTQPGTDLRADRDLHSAPAVSLCGCNLRVLYQRAEAEKQQNISPLVRERGPQRVAAHITGTRGRSNTLSSPNSKNEKALGRKINSWESSRSGHSFLSNLHLRNGELVIHEKGFYYIYSQTYFRFQEEIKENTKNDKQMVQYIYKYTSYPDPILLMKSARNSCWSKDAEYGLYSIYQGGIFELKENDRIFVSVTNEHLIDMDHEASFFGAFLVG

SEQ ID NO: 8 - protein, 178 aa, homo sapiens
KEKQQNISPLVRERGPQRVAAHITGTRGRSNTLSSPNSKNEKALGRKINSWESSRSGHSFLSNLHLRNGELVIHEKGFYYIYSQTYFRFQEEIKENTKNDKQMVQYIYKYTSYPDPILLMKSARNSCWSKDAEYGLYSIYQGGIFELKENDRIFVSVTNEHLIDMDHEASFFGAFLVG

SEQ ID NO: 9 - DNA, 2301 bp, homo sapiens
aaggcaagagatctaggacttctagcccctgaactttcagccgaatacatcttttccaaaggagtgaattcaggcccttgtatcactggcagcaggacgtgaccatggagaagctgttgtgtttcttggtcttgaccagcctctctcatgcttttggccagacaggtaagggccaccccaggctatgggagagatttgatctgaggtatgggggtggggtctaagactgcatgaacagtctcaaaaaaaaaaaaaaaagactgtatgaacagaacagtggagcatccttcatggtgtgtgtgtgtgtgtgtgtgtgtgtgtgtgtgtgtgtggtgtgtaactggagaaggggtcagtctgtttctcaatcttaaattctatacgtaagtgaggggatagatctgtgtgatctgagaaacctctcacatttgcttgtttttctggctcacagacatgtcgaggaaggcttttgtgtttcccaaagagtcggatacttcctatgtatccctcaaagcaccgttaacgaagcctctcaaagccttcactgtgtgcctccacttctacacggaactgtcctcgacccgtgggtacagtattttctcgtatgccaccaagagacaagacaatgagattctcatattttggtctaaggatataggatacagttttacagtgggtgggtctgaaatattattcgaggttcctgaagtcacagtagctccagtacacatttgtacaagctgggagtccgcctcagggatcgtggagttctgggtagatgggaagcccagggtgaggaagagtctgaagaagggatacactgtgggggcagaagcaagcatcatcttggggcaggagcaggattccttcggtgggaactttgaaggaagccagtccctggtgggagacattggaaatgtgaacatgtgggactttgtgctgtcaccagatgagattaacaccatctatcttggcgggcccttcagtcctaatgtcctgaactggcgggcactgaagtatgaagtgcaaggcgaagtgttcaccaaaccccagctgtggccctgaggcccagctgtgggtcctgaaggtacctcccggttttttacaccgcatgggccccacgtctctgtctctggtacctcccgcttttttacactgcatggttcccacgtctctgtctctgggcctttgttcccctatatgcattgcaggcctgctccaccctcctcagcgcctgagaatggaggtaaagtgtctggtctgggagctcgttaactatgctgggaaacggtccaaaagaatcagaatttgaggtgttttgttttcatttttatttcaagttggacagatcttggagataatttcttacctcacatagatgagaaaactaacacccagaaaggagaaatgatgttataaaaaactcataaggcaagagctgagaaggaagcgctgatcttctatttaattccccacccatgacccccagaaagcaggagggcattgcccacattcacagggctcttcagtctcagaatcaggacactggccaggtgtctggtttgggtccagagtgctcatcatcatgtcatagaactgctgggcccaggtctcctgaaatgggaagcccagcaataccacgcagtccctccactttctcaaagcacactggaaaggccattagaattgccccagcagagcagatctgctttttttccagagcaaaatgaagcactaggtataaatatgttgttactgccaagaacttaaatgactggtttttgtttgcttgcagtgctttcttaattttatggctcttctgggaaactcctccccttttccacacgaaccttgtggggctgtgaattctttcttcatccccgcattcccaatatacccaggccacaagagtggacgtgaaccacagggtgtcctgtcagaggagcccatctcccatctccccagctccctatctggaggatagttggatagttacgtgttcctagcaggaccaactacagtcttcccaaggattgagttatggactttgggagtgagacatcttcttgctgctggatttccaagctgagaggacgtgaacctgggaccaccagtagccatcttgtttgccacatggagagagactgtgaggacagaagccaaactggaagtggaggagccaagggattgacaaacaacagagccttgaccacgtggagtctctgaatcagccttgtctggaaccagatctacacctggactgcccaggtctataagccaataaagcccctgtttacttga

SEQ ID NO: 10 - DNA, 2301 bp, homo sapiens
aggaattgaactcagctctgccccaagcggacctaatagacatctacagaactctccaccccaaatcaacagaatatacatttttttcagcaccacaccacacctattccaaaattgatcacatagttggcagtaaagctctcctcagcaaatgtaaaggaacagaaattataacaaactatctctcagaccacagtgcaatcaaattagaactcagaattaagaatctcactcaaaaccgcacaactacatggaaactgaacaacctgcttctgaatgactactgggtacataatgaaatgaaggcagaaataaagatgttctttgaaatgaacaagaacaaacacacaacataccagaatctctgggacgcattcaaagcagtgtgtagagggaaatttatagcactaaatgcccacaagagaaagcaggaaacatccaaaattgacatcctaacatcacagttaaaagaactagaaaagcaagagcaaacacattcaaaagctagcagaaggcaagagataactaaaatcagagcagaactgaaggaaatagagacacaaaaacccttcaaaaaattaatgaatccaggagctggttttttgaaaggatcaacaaaatagatagaccactagcaagactaataaagaaaaaaagagagaagaatcaaatagacacaataaaaaaatgataaaggggatatcaccaccgatcccacggaaatacaaactaccatcagagaatactacaaacacctctacgcaaataaactagaaaatcaagaagaaatggataaattcctcgacacatacactctcccaagactaaaccaggaagaagttgaatctctgaatagaccaataacaggatatgaaattgtggcaataatcaataccttaccaacaaaaaagagtccaggaccagatggattcacagccgaattctaccagaggtacaaggaggaactggtaccattccttctgaaactattccaatcaatagaaaaagagggaatcctccctaactcattttatgaggccagcatcattctgataccaaagccgggcagagacacaaccaaaaaagagaattttagaccaatcaatatccttgatgaacattgatgcaaaaatcctcaataaaatactgccaaaccaaatccagcagcacatcaaaaagcttatccaccatgatcaagtgggcttcatccctgggatgcaaggctggttcaatatacgcaaatcaataaatgtaatccagcatataaacagagccaaagacaaaaaccacatgattatctcaatagatgcagaaaagacctttgacaaaattcaacaacccttcatgctcaaaactctcaataaattaggtattgatgggacgtatttcaaaataataagagctatctatgacaaacccacagccaatatcatactgaatgggcaaaaactggaagtattcactttgaaaactggcacaagacagggatgccctctctcaccactcctattcaacatagtgttggaagttctggccagggcaattaggcaggagaaggaaataaagggtattcaattaggaaaagaggaagtcaaattgtccctgtttgcagacgacatgattgtatatctagaaaaccccattgtctcagcccaaaatctccttaagcagataagcaacttcagcaaaatctcaggatacaaaatcaatgtacaaaaatcacaagcattcttatacaccaacaacagacaaacagagagccaaatcatgagtgaaatcccattcacaattgctttaaagagaataaaatacctaggaatccaacttacaagggatgtgaaggacctcttcaaggagaactacaaaccactgctcaatgaaataaaagaggataaaaacaaatggaagaacattccatgctcatgggtaggaagaatcaatatcatgaaaatggccatactgcccaaggtaatttacagattcaatgccatccccatcaagctaccaatgcctttcttcacagaattggaaaaaactatttttagttcatatggaaccaaaaaagagcccgcattgccaagtcaatcctaagccaaaagaacaaagctggaggcatcacactacctgacttcaaactatactacaaggctacagtaaccaaaacagcatggtactggaaccaaaacagagatatagatcaatggaacagaacagagccctcaaaattaatgccacatatctacaactatctgatctttgacaaacctgagaaaaaccagcaatggggaaaggattccccat

SEQ ID NO: 11 - DNA, 2024 bp, homo sapiens
aaggcaagagatctaggacttctagcccctgaactttcagccgaatacatcttttccaaaggagtgaattcaggcccttgtatcactggcagcaggacgtgaccatggagaagctgttgtgtttcttggtcttgaccagcctctctcatgcttttggccagacagacatgtcgaggaaggcttttgtgtttcccaaagagtcggatacttcctatgtatccctcaaagcaccgttaacgaagcctctcaaagccttcactgtgtgcctccacttctacacggaactgtcctcgacccgtgggtacagtattttctcgtatgccaccaagagacaagacaatgagattctcatattttggtctaaggatataggatacagttttacagtgggtgggtctgaaatattattcgaggttcctgaagtcacagtagctccagtacacatttgtacaagctgggagtccgcctcagggatcgtggagttctgggtagatgggaagcccagggtgaggaagagtctgaagaagggatacactgtgggggcagaagcaagcatcatcttggggcaggagcaggattccttcggtgggaactttgaaggaagccagtccctggtgggagacattggaaatgtgaacatgtgggactttgtgctgtcaccagatgagattaacaccatctatcttggcgggcccttcagtcctaatgtcctgaactggcgggcactgaagtatgaagtgcaaggcgaagtgttcaccaaaccccagctgtggccctgaggcccagctgtgggtcctgaaggtacctcccggttttttacaccgcatgggccccacgtctctgtctctggtacctcccgcttttttacactgcatggttcccacgtctctgtctctgggcctttgttcccctatatgcattgcaggcctgctccaccctcctcagcgcctgagaatggaggtaaagtgtctggtctgggagctcgttaactatgctgggaaacggtccaaaagaatcagaatttgaggtgttttgttttcatttttatttcaagttggacagatcttggagataatttcttacctcacatagatgagaaaactaacacccagaaaggagaaatgatgttataaaaaactcataaggcaagagctgagaaggaagcgctgatcttctatttaattccccacccatgacccccagaaagcaggagggcattgcccacattcacagggctcttcagtctcagaatcaggacactggccaggtgtctggtttgggtccagagtgctcatcatcatgtcatagaactgctgggcccaggtctcctgaaatgggaagcccagcaataccacgcagtccctccactttctcaaagcacactggaaaggccattagaattgccccagcagagcagatctgctttttttccagagcaaaatgaagcactaggtataaatatgttgttactgccaagaacttaaatgactggtttttgtttgcttgcagtgctttcttaattttatggctcttctgggaaactcctccccttttccacacgaaccttgtggggctgtgaattctttcttcatccccgcattcccaatatacccaggccacaagagtggacgtgaaccacagggtgtcctgtcagaggagcccatctcccatctccccagctccctatctggaggatagttggatagttacgtgttcctagcaggaccaactacagtcttcccaaggattgagttatggactttgggagtgagacatcttcttgctgctggatttccaagctgagaggacgtgaacctgggaccaccagtagccatcttgtttgccacatggagagagactgtgaggacagaagccaaactggaagtggaggagccaagggattgacaaacaacagagccttgaccacgtggagtctctgaatcagccttgtctggaaccagatctacacctggactgcccaggtctataagccaataaagcccctgtttacttgaaaaaaaaaa

SEQ ID NO: 12 - DNA, 2421 bp, homo sapiens
caccctcatgagccccgggtacgtttaactattgagggccaggaaattgccttcctcctggacactggcgcagccttctcagggttaatctcctgtcctggatgactgtcttcaaggtccgttaccacccgaggaatcctgggacagcctataaccaggtatttctcccacatcctcagttgtaattgagagactttaatcttttcacatgccttttttgttattcctgaaagtcccacacccttattaaggagggatatattagccaaggctggagctattatctacatgaatatggggaaaaagttacccatttgctgtcccctacttgaggagggaatcaaccctgaagtctgggcattggaaggacaatttggaagggcaaaaaatgcctgcccagtccaaatcaggttaaaagatcccaccacttttccgtatcaaaggcaatatcccttaaggcctgaagctcataaaggattatagaatattgttaaacatttaaaagctcaaggcttagtgaggaaatgcagcagtccctgcaacaccccagttctaggagtacaaaaaccaaacagtcagtggagactagtgcaagatcttagactcattaatgaggcagtaattcctctatatccagttgtacccaacccctataccctgctctctcaaataccaggggaagcagaatggttcacggttctggacctcaaggatgccttcttctttattcccctgcactctgactcccagtttctctttgcttttgaggatcccacagaccacacgtcccaacttacacagatggtcttgccccaagggtttagggatagccctcatctgtttggtcaggcactggcccaagatctataggccacttctcaagtccaggcactctggtccttcaatatgtggatgatttacttttggctaccagtttggaagcctcgtgccagcaggctactctggatctcttgaactttctggctaatcaagggtacaaggtgtctaggtcgaaggcccagctttgcctacagcaggttaaatatctaagcctaatcttagccaaagggaccagggccctcagcaaggaatgaatacagcctatactggcttatcctcaccctaagacattaaaacagttgcggggattccttggaattactggcttttgctgactatggatctccagatacagcgagacagccaggcccctctatactctaatcaaggaaacccagagggcaaatactcatctagtcgaaagggaaccagaggcagaaacagccttcaaaagcttaaagcaggctctagtacaagctccagctttaagccttcccacaggacagaacttctctttatacatcacagagagagccaagatagctcttggagtccttagactcgtgggacaaccccacaaccagtggcatacctaagtaaggaaattgatgtagtagcaaaaggctggcctcactgtttaagggtagttgcagcagcggccgtcttagcgtcagaggctatcagaataatacaaggaaaggatctcactgtctggactactcatgatgtaaatggcatactaggtgccaaaggaagtttatggctatcagacaaccgcctcttagatgccaggcactactccttgagggactggtgcttaaaatatgcacgtgcgtggccctcaaccctgccacttttctcccagaggatggggaaccaattgagcatgactgccaacaaattatagtccagacttatgccgcccgagatgatctcttagaagtccccttaactaatcctgaccttaacctatataccgacggaagttcatttgtggagaatgggatacgaagggcaggttacgccatagtgatgtaaccacacttgaaagcaagcctcttcccccagggaccagtgcccagttagcagaactagtggcacttacccgagccttagaactgggaaagggaaaaagaataaatgtgtatacagataacaagtatgcttatctaatcctacatgcccatgctgcaatatggaaagaatgggagttcctaacctctgggaacccccgctggatgccacagggaagttatggagttattgcacatggtgcaggaacccaaagaggtgggagtcttacactaccaaggccatcaaaatgggaaggagaggggagaacagcagcataagcggctggcagaggtagggaaagaccagcaagaaggaaagagagaaagagaaagtcagagaaagagacagagagaggaagagacagagagacagaacgttaaagagggtgtcagaaacagagacaaacaaaaggagtcagaaagaaggacagacacagaaagtcaaagagagagttaaaaagagaggaagagacaaagaagtcgaagagagaaagagagagatggaagt

SEQ ID NO: 13 - DNA, 2421 bp, homo sapiens
ctttgcagataaatatggcacactagccccacgttttctgagacattcctcaattgcttagacatattctgagcctacagcagaggaacctccagtctcagcaccatgaatcaaactgccattctgatttgctgccttatctttctgactctaagtggcattcaaggtaaggaacatcaaaggatacttaatttgtaaaatgagaaataggaataggtataaattctaaaaatacagaaataatgtatttgtaaaagtttcactgcatgcttataaataagagggaaataaatagagattccctcagatcataaaacttatatgaattgaagtgagagaaacaaatagaataagagaaagagaaggaaaaagggaaggaggacagaagagatggggaagagggaggatagagagagaaaatgtgagggaatgcggacagagatgagatacagatacttccttacctaactaagctcaatgaaccacatgaactgtgcttaagggtttgactttataatcaacaagctgcaattcttttcttccagataatcaactctttaatcatttacagttgtgttatgatgtgatccattcctcctcagattaagtgactatttgctgatatggggatataggttctgctaaataccaccagtctacattaaatgcctaaaatgaacactgtgctaaccttctctgctgttcctcttttcctacaggagtacctctctctagaactgtacgctgtacctgcatcagcattagtaatcaacctgttaatccaaggtctttagaaaaacttgaaattattcctgcaagccaattttgtccacgtgttgagatcatgtgagtgaaatcccatctgattatcacttccctggttgtaattatatactgtattaaatatgtaatgataataaaaaaagatcagtaaagggtttgtgatgattctaaaactaatgtacagcaaacaaaaacatgcagagtgaaacttaaatgtctgacttcagaactgcgtatgccatctgttttattgacccaacacagttttaaatattttcatccctatttatttctacagtgctacaatgaaaaagaagggtgagaagagatgtctgaatccagaatcgaaggccatcaagaatttactgaaagcagttagcaaggaaaggtaggtttgctgttgcctgcagaagaattgctctttaggaaacggcaatcttgggagtcagaaatacttgcattgtggtttgctgtgcaatcgctggtttaaaagtatgttaccaccacgccctcccctacctccatttatttaaatgctgaggcaccatcttgtgtgataagtatcagaagttaccctgattaccagtcaaccttgaagtacagctataactatctaagcaaaactgacaacattttccccaagtctttcatggttgaaaaaagcaacccctataatccataatgaatgcatagcagcaggaaagctcagttatctattctatgaactcggtactttccaaacacaacccaatctgaagccagagtcagactatcacacttttatatcccctttctcttcttacaggtctaaaagatctccttaaaaccagaggggagcaaaatcgatgcagtgcttccaaggatggaccacacagaggctgcctctcccatcacttccctacatggagtatatgtcaagccataattgttcttagtttgcagttacactaaaaggtgaccaatgatggtcaccaaatcagctgctactactcctgtaggaaggttaatgttcatcatcctaagctattcagtaataactctaccctggcactataatgtaagctctactgaggtgctatgttcttagtggatgttctgaccctgcttcaaatatttccctcacctttcccatcttccaagggtactaaggaatctttctgctttggggtttatcagaattctcagaatctcaaataactaaaaggtatgcaatcaaatctgctttttaaagaatgctctttacttcatggacttccactgccatcctcccaaggggcccaaattctttcagtggctacctacatacaattccaaacacatacaggaaggtagaaatatctgaaaatgtatgtgtaagtattcttatttaatgaaagactgtacaaagtagaagtcttagatgtatatatttcctatattgttttcagtgtacatggaataacatgtaattaagtactatgtatcaatgagtaacaggaaaattttaaaaatacagatagatatatgctctgcatgttacataagataaatgtgctgaatggttttcaaaataaaaatgaggtactctcctggaaatattaagaaagactatctaaatgttgaaagatcaaaaggttaataaagtaattataactaaga

SEQ ID NO: 14 - DNA, 2421 bp, homo sapiens
agatgacttttttctatttatatttaataagatgatgaacccttcttgcattcccgaaataaacctcaactgttacagtgttttattcttttaatatgtacgaagtacatgttaagcaagttatttcctaagcagccccacaaactgggcactactaccatcctgctctgcccctccctcactctacttcagccacttcagccacaatggcctctcctcactgcccctctgatgcaccaagcttgttctcacctcaggaatgtgcaacacctgccagacttgctgttccccggagcctccatccccagatatcctcatatatcatcctcctcttcatttgtgtctctgcttacatatgacctatttacagaagcctttcctgtctaccccccatgaaatagaaatcgcattccaatcttgtctctaccccaatgctgtttcattttgtctgtagcaattgtcatcatctcatatatattcacatgtggaaaatacacaaaatgtttaacttcttttaatttacattccatttccccatgaattgaagctccatgacagcggagatttttctctgctttccctgttgctcacttcccagcaccaagagcaggcctggcacatgggaagtacttactatttattgaatggatgaatgaacaaatgaatgaatggatacttattttacacataagaaaactgaagcttatagaaattaagtaactaaaatcacacagaagcacagctgaaactaaaacctacgtctaactttcaattcctgacccttaaccattaaaacaaatgacaggtgactttaggccactgaaaatgctcatataatcttatgaattctaaagcacaagttaatcacaccattgattgaaagtctgaggaatactgtatagacaagcccctgtacaaggtaagcaaaagaatcagaggatggcctccaaagaattccctggacattatgggaattacattgttagccttcctactgatacccataagcctcacagcaagcatcatgaagctgtgaccttcatctgcacatgcccttgtatacccaaaagataaaactggatgcttcagggccgaatggccaataaacacgtgtttattactggcatgggcagacacacatactgaaagtaccatttcccagcggactagccatattatgatcagtacagacactaaagatttagctttgaaaaaactatttgctcttccaaagctgaagaatcttctgtgatttcaacaggcaagttacagtcaggtattcttaatgttcttttcctcctctctcactgggatactttctttccttcagacaacgtcaagcgaaaaacaaaatttcacaaatctccatttctgacactaaacagtacagtatctttattttttttataatttaatcaaaccctgtattttagaactgtggggctgatccaacattgcaatgtgtcacatttaattccatcaatgtaaagcataatgagcaaagattaaggtagtgaggcataactaaatgttttgaacctgtgaatttcaaaagcaaggcccatttgtgttattttctaaatagtaaataaaatcattttccaacatttcactatcaaattacagtaatttttccaccagtacacacttgaggaaagccacaaaaagacttttccaacagttcattctgttattgctcataaccttctaaatacttctcctcattggcttctattcaaaggtaaatggaaagcagtaaaatttatggaaaatatattcaactgcttaaaatacatcaaccaaaaaaaagattttagagctgtattatgagttgtgaaattgcattgccttcacttacctttcagtttcactggtaggtaacaaaactgacagactggtcaagttccaaaacatcccctatatagagcctgactcttccatctcaaattctcaccttggtcaaggccagagtaaacacctgtccttcacatttttacacaacatcactttgtatgctacaaatataagctttcataccagggaggaagcaaattccaggacactggaaacatttctgctctcttaaaccagtctgttgattgttcccttgactttctcagctgtcaggatagtgaaaggaggaaaactgcaaaactgtaaagtataacctgataagtttgccctttaagcttttcacacagagagaggtaaaataaaactcaagtctaaggtttaaaattgagctatgaatattatattctagcactagacaaaaatgttgcaagattttaataaaataagattattaaaatcaatttttacatttcatgggccaaggagagacatcaaagaatgtttaactaacattttaaagatactatactttataaagttaagaagaaaaatgacaactgcaccagt

SEQ ID NO: 15 - DNA, 1227 bp, homo sapiens
ctttgcagataaatatggcacactagccccacgttttctgagacattcctcaattgcttagacatattctgagcctacagcagaggaacctccagtctcagcaccatgaatcaaactgccattctgatttgctgccttatctttctgactctaagtggcattcaaggagtacctctctctagaactgtacgctgtacctgcatcagcattagtaatcaacctgttaatccaaggtctttagaaaaacttgaaattattcctgcaagccaattttgtccacgtgttgagatcattgctacaatgaaaaagaagggtgagaagagatgtctgaatccagaatcgaaggccatcaagaatttactgaaagcagttagcaaggaaaggtctaaaagatctccttaaaaccagaggggagcaaaatcgatgcagtgcttccaaggatggaccacacagaggctgcctctcccatcacttccctacatggagtatatgtcaagccataattgttcttagtttgcagttacactaaaaggtgaccaatgatggtcaccaaatcagctgctactactcctgtaggaaggttaatgttcatcatcctaagctattcagtaataactctaccctggcactataatgtaagctctactgaggtgctatgttcttagtggatgttctgaccctgcttcaaatatttccctcacctttcccatcttccaagggtactaaggaatctttctgctttggggtttatcagaattctcagaatctcaaataactaaaaggtatgcaatcaaatctgctttttaaagaatgctctttacttcatggacttccactgccatcctcccaaggggcccaaattctttcagtggctacctacatacaattccaaacacatacaggaaggtagaaatatctgaaaatgtatgtgtaagtattcttatttaatgaaagactgtacaaagtagaagtcttagatgtatatatttcctatattgttttcagtgtacatggaataacatgtaattaagtactatgtatcaatgagtaacaggaaaattttaaaaatacagatagatatatgctctgcatgttacataagataaatgtgctgaatggttttcaaaataaaaatgaggtactctcctggaaatattaagaaagactatctaaatgttgaaagatcaaaaggttaataaagtaattataactaagaaaaaaaaaaaa

SEQ ID NO: 16 - protein, 98 aa, homo sapiens
MNQTAILICCLIFLTLSGIQGVPLSRTVRCTCISISNQPVNPRSLEKLEIIPASQFCPRVEIIATMKKKGEKRCLNPESKAIKNLLKAVSKERSKRSP

SEQ ID NO: 17 - DNA, 5687 bp, homo sapiens
ctctctggttgcccttaacattttttccttcatttcaactttggtgggtctgatgattatgtgtcttggggttgctcttctcgaggagtatcttagtagtattctctgtatttcctgaatttgaatgttggcctgtctttctaggttggggaagttctcctggataatatcctgaagagtatttttcaacttggttctattctccttgttactttcaggtacaccaatcaaacgtagatttggtcttgtcacatagtcccatatttcttggaggttttattcgttcctttttattcttttttctctagttttgtcttctcgctttatttcactaagttgatcttcaatctctgatatccttgcttctgcttgattgattcagctatcccccgctcgatattacaaaccatgtcacgaggcgtggacaccccccatgatatggggagtattatcacccccctcttcccccactggatattacaaaccatgtcatagggaggtggacatcccccacaatatgaggagtaatatcacacccctttccccgcagtggatattatgaaccatgtcacaggcggttaaacacccccaacgatatggggagtaatatcacactcctctcccccctggatattacgaaccatgtcatggggggtggacaccctttgcaatatggggagtaaaatcacccccctctcccccaactggatattatgaaccatgtcacagtgggggaaaaatcctctgtgatatgcagagtaatatcaccccactctcaccacctggatattacgaaccatgtcacaggggggtggacaccccccaagatgggggagtaatatcacctcactctctgccaccagatattacaaactgtgtcacaggggggtgaacaacccccacaatatggggagcactatcacccccctcccccagggtattatgatccatgtcacaggggggtggataccacccactatatggggagtaatatcacctttctctcccgccctggtttttatgaaccgtgtcacaggggggtggacaccccttgcgatatggggagtaatatcacccccctctccaccatctggatattacgaaccatgtcacaggggggtggacacccctgcgatatggggaggaatatgcccctctccccacctggatattacaaatcatgtcacgggggacggacatcccccacaatatggggagtaatatcaccacactctcccctgctggatattacgaaccatatcacaggcggctggagacacaaggcattaacaatatttcgagtaatattatctttccctttgaacattatgaacaatatgacagaggggtgtacacctcctgcgatattgggagtaatgtcatcccctcccccactggatattaggaaccatattactgggggatgtattcccccttctagattgggaggaagatcatacttgccctccctgaatatttgaaacaatatcataggggtttgtacacttttacgatattgggagtaatatcatcctttctccccctggaaattaggaacaatatcacaggggtggtgtacacccctgcaatatttagggtaatattattgtcttctcccctcgatattaggaacaatattacaaggacggtgtaaagtacctgccaaattgggaaaaatactatcctctccctcttgtatattagaaacaataacacagggggaatgtacacccactgccatattgggagtaatatcatactcgccccatcccccagatattaggaacaatatcacagcaggggtgtacacttttacgatattgggagtaatatcatactctctccccctggaaattaggaataatatcacagagatggtgtagaccctctgcaatacttaggataatattatcatctcccccctcgatattaggaacaatattacggggagtgtaaattacctgccaaattggaggtaatcctctcctctctctccctgtattttagaaaatataacacacaggaaatgtacaacactgcgatattcggagtaatatcttcttctccccacctggatattaggaacaataacacggacggggcgtacacccctcgcgatattgaatgtaatgtcatcctctccctccctttatattacgaacaatatcacaggggggtgtacaacccctgcaatattggaagtagtatcatccattctcccatgaatattaggaacaatatcacaggggtagagtacaccctctgcaatttcgggagtaacatcatcctctcgttccctggatattataaacaacaccacgggggggtgggggtgtacacacccttcgatattgggagtaatataatcctttccctccctatatattagaagcaatatcacaggggttggtgtaaacttcttgcgatatggggattaatatcacccccctctcctgccctggatattatgaaccatatcacagggaggtggacacactttgcgatatggggagtaatatcacgcccctctcccccccgatattacgaaccatatcacaagggagtggaccccccccacgatatggggagtaatatcacccccctctcccgccctggatattacgaaccatatcacagggggatggacaccccccgcgatgcggggagtaatgtcacccccttctgccccctaggatattacgaaccatatcatggacaccctccacgatattggaaataatatcatcctctcccccttggatattaggaacaatatcacagggggttgtacacctcctatgatattggaagtaatatcatcctctccctcctggatattagcaacaatatcacagggagtgtgtacaaccccagcgatatttggagtaatatcaccctctcaccccatggatatgagaaacaatatcacaggggaggtgtacatcccacgtgatattgtgtgtaatatcattcttccccaacccctgcaatattgtggtgtaatataattctctcccttcctggacattatgaacaatatcactactaggtgatacattaggagtaatgtatccataggatattatgaggaatatcacagggtgtacacccactgtgatattagaggtaatatctccctaaaatattaagaagaatatcttacacccactgtgactttagaagtaatatctccctaaaacgttacaaataacatcgcagggtgtacactcacagtgatattaggagtaatatctccctagaatattacaaatacacatggtgtaaacccactgtgactttagaagaactatctccctaaaataatacaaaaatatcgcagtgtataccataatatcccctagaatatcataaataatatcacagggtgtacacccactgtgataataggaataataccaccccaggatattatgaataatgtcacaggctgtacacccactatgacattaggagtaatatctccctaggacactatgaataacatcacagattttacacccatggtgtgcacccactatgatattaggagtaatatctgcacaggatataacaaataatagtacagggtgtacacatatgatatacacccactgtgatattaggagaaatatatccctaggatattatgaataacctctcagagtacacacacatggtatacaccctctgtggcattaggaacaataactttctaaaacattacgaataacatcacagaatgtacacacatggtttacacccactgtgacaggtgcaatatctcccttggatattatgaataacaacaaactatcactgtcatattaggagtaatttctccctagaatattacaaataacatcacagggtgttcatttatggtgcacacccactgtgatattaggagtaatatctccctaggatattacttttcatataaaagtgtgtacatccactgtgatattgggaaaaatatttctctaggatattatgaataatatcacagagcgtacacccactgtgatattaggagtaataattccctgggttattatgaataatatcacaggatgtacaaccactgtgatattaggagcaatatcttcctaggatattacaaataatatcacagggtgtacacccactgtgatattaaagtaatttttaggttattgtgaataatatcaccaagtgtacaaacatggtgtacactcactgtgatatcaggagtaatatctcagtaaaatattatgaataatatcacagggtatacacccactgtgatattagcagtagtatctttgtaggatattacaaataatatcacagggtgtatgcccactatgacattagaagcaatatctccctaggatatcaaaaataatatcacagggtgtacaacttctacatcccaggttctaagggattctcctgcttcagcctcctgagtggctgggattacagatgcccaccaccacacctggctaatttcgtattttcagtagagatggggtatcaccatgctggtcaggctggtctggaacttctgacctcaggtgatccaccagcctcggccttccaaagtgctgggaatacaggtgtgagccaacgtgcttggcagagagttatatattaaataaatctggaaacatagctcccatgtttgagtgtgcatttacttttatgaagaaattatgtcagaaaacctaaggatgataataaatatgaaaagtaactggcatgtaaaaaggtcttttgattaagaactataaggttcgatttcatttttagataacgtgatcctagctcttgtatagtgcttataaatattctacatcaaaggaatttgttgcacagtgtcagaataaaataaagtgtatttcactgcttcttaatttttaaattagactgagtttgttttcctagagagagaagaacattttttattttttctgaaaagagtaggccatattttactgagatcttagatttgttatatattaggttttggtcttctaacattctccagtggattttctctaaagtaggtatgcacagaaagagttgaatagcaaaaaagtaaatcatgtaataattctgagatttttgggtttgtcacaactgagaaatattgctgagggtgtatggtcctcaagtgtgaaaatgttccttgtgaattgcttgtatccgaaatatacacacaacattaagtcctggtttttatcttttattttttccaatccttttttcttctcaaggtgtccaagtcacacagagccacagaatctcacaggtgtctcagaattcctcctcctgggactctcagaggatccagaactgcagccactccttgctgggctgttcctatccatgtgcctggtcacgatgctggggaacctgctcatcatcctggccgtcagccctgactcccacctccacatccccatgtacttcttcctctccaacctgtccttgcctgacattggtttcaccttggccacggtccccaagatgattgtagacatgcaatcacatagcagagtcatctcccatgcaggctgtctgacacagatacctttctttgtcctttttgtatgtatagatgacatgctcctgactgtgatggcctatgactgatttgtggccatctgtcaccccctgcactacccagtcatcatgaatcctca

SEQ ID NO: 18 - DNA, 5687 bp, homo sapiens
attgaattttatctcagagcccacatgaagcaggatcaaagtcagtacacatgaaaactagagcccaaagactataaagcatgaaataaggatttaagctaaccctatcttgtaaggggtttgtaaagcccagcttgcatctgagctacactagcaccaggacagccactcagtaatggggtttctcaaggttattgcttttcattcagttgaaatgagagtcatttcttacccttatgccctgtgagatttcactggaggttgttcactgaaacattttcatatcattgcatcaaccctcttgaactcactgtgcctgcccccagttcagtctgtgactcacaagtaccctgcagcaaaagaaatccaatagagggcaaatccctcaccttaccttcctttctaagacctttgatgttctcatgtgtcatttcataattgggattgtcaattagtcgcctcatctctggtcctcactttcctctctcccagccaaactcaaccttcagcccacacaatggaattcaacaaaatgaggtaacagttttctgtgtgagtcactctgggcaactctgttcacagagcactgtgaggtgagcagccagaacccaggcaagtgtttcagccatccaagaactggcaggcagcccaagagacactctcacctgatgacagactagcaggatgagtcctggaggaaatggttcccaacagctgcagaaggagtctcttggctcatgcacagcaatgctcttctcaattaaaaacgttgtcattattgacactgcagtgtaaaatccttttacactgtgctcacatttctacaggccttcacctgctctgcccattaaagacaagacccttccatgagatgatgacatctctaagttactgttccacccaaacagtcctatataatgaagagaaaaattttgctggccctcaaaaggcaaacacaaggagaaagatttccacaagctgtttctctttgctgagcacttagaggaaaactgtaagtggttggaagaaggctttgttttctacaagacttttagttattcctcagaaattttcctgcttattcccagaggaggtcatctcttagatgctgtcagtcagatagggattggcagccaagcagaggtgctcagagaggtttccaactaatgtggccagcggaaaactgccaaagaagcagggatccttaggacaaataaactggaagatattttggggataaaaataaatccttttgaaaatgaaagatggagagatgctgtatatacaaattgccctgttctgaacaatgttgtcactaggactggccctggagaccaatgatacaaaccaaaatgttctcagacatgctttgatggtctttttctccaaagttatctattctgtttccatttcattctcacaggacttgccatggggttctcataagatttcacattggtcataatccaggtggccctggactgcaacctctgagttggcaacatcagaataggaattacgaaaaaccaatttaaagttaaatacagacacaggcaaaagagagatgggttgtcgaagctagtgcctaggtggacactgcctcacatttttaattccagaagccatcagtactgagtgtcagatctcattagtcaaacacagtgatcaggaatcctgttttcctggaggatttccttgagggagggaccactcaagagtctgaaatatttcacgtcatagagtatggatctcaccccaacacccaatcagaaaatagggagaactggaaaccaaaattccccctcccgctgtggaaggatgaaaaccagagtgttggagttctgtcctgataatggagcagacagctaggcagcaatcaatgagggccagtacaggaattcagtgctaagtattgggtcataacagaagtagggaaggtattaatccagtgctatatgaggatcctgggacactggctcctagtaatctagttataactattagcaaaaaagaaaaaaaaaatcagtgatgtgaagagatggcctaaaggagctccagcaatatagctaagcagctggcaagtggtctgaggagcattgcaattccaggcctcctaaggtggcagtacgggcactggtaagacattctgctgtggtgaaactagtttaccatagaggattcacaattaaaataggcaaacaggaaatgcaagacagaggctaacaaagggttttttttttggtgggggggagttgtttgtttgtttgtttgttttctgagacggagtcttcctctgttgcccaggctggaatgcagtggcacgatctcagctcactacaacctctgcctcccaggttcaagcagttcttctgcctcagcctcccaggttcaagcagttcttctgcctcagcctcccaagtacctgggactatagctgtgtgccaccacattgactaatttttgtacttttagtacagactgggtttcaccatgttggccaggctggtgtcgaactcctgacctcaagtaatccccccgccttggcctcccaaagtgctggaattacaggcatgagccaccacacctggccagtttttggtaattcttaaagaactcaatgagcaacactcaaacaaccataaagactatagagctcatggttgaattttagatagctaaacagacaggagtttttgtaagttttgtaagtcttgctcatccttccctcttccatcctctatctcaactattctgtctaccattaaagcaccttagaccttgagtttggcaatgcaacaagtgtgtgctcaacacgaaataggtaattcaatagcaaagccctaaaacagcctggcttgattatttctcagggcatgcagttcctttgaagcaggatcattttaataataataataatagaaataataatagaaattgaagacaattatttcacaatttccatacacctaagagctatacatatgaatgataatgcataattgtaaagcatgcatattacaggtaataaatatgttagctaattataaacaatgcccattttcatatagtttatccttgccaaataaaactgtaaaaaaaagacacctttcaaatgctgctaaggagtaatacctgaatgaggttgatttaatggagtcttagttcctgcatgtgttctaattgaatagactatgtagtaattcccttacatacccatccatgtccaagaacagtgaagatctttatttaatatgaattattgcagatgattagcacagtctagccaaaccattccagtaattgtttttacttgttatattaatatataaattctcaaaggatataacagtgatgttgggtgaatttcactgaatgatagctcaaacacctgaaatattgactaagaaaactaatttatcaatactgataatcaattttaatatgttaattgattgtaatacaggattctgtggttcaaaaaaaaagaacaagcaaaaaaactttcttccatttccaaataccaattaatagatctctacttccccttggatttcttcttaccacctaccacctccaatcttcattctttcctcacaaactaaacataaaagttacctacaaagcatagaatctgtgttaaaggatattcttgcttgttttaagtccaaaattaaacagctctgaattattaaaaagcacatgaattcaaatgtcctattctaataagaaaatggtttacatttctctatgttcaaggaaaaaaatagtcaagggtgtacaagtggggtaaaaattatttccagtaggttatgtgatttaagttatagaaacgaaccaggcaattcaattaaatgtcatggaaagtaggttttttcttttcctctttttttctaatatgtacactttgtgagaagataaatccatagtgtgataatttgtccactgggtccatcagacactggagacagcttcctaagaattataaggcttctaaaggcttctaaagcctaaattgcctagagcattttgtgtgccaggcactttgctaggtgccctagggatgcaagaagtataaatgttttatgagaatacaggctggaaatgtattcttgattattcctgtggaatttctaggcagaaaagagtctaatggggtataggtatattttctcaacacaattttctgagcctttaccagatgcagttctatggtttgaatgtgtccctcagagtttgtgtgttggaaacttaatccccaatgcaataatgttggtgaggcctaatgaaagcctaataatgtaggtgaggcctaatgagagctgtttagaccatgaaggctcttccctcatggatggattaatgctgttatggtgggaatgggttcattattactggggtgggttcataataaaaagatgagtttggcctgctattctctctctttctcatcctctcttccaccatgggatgacacagcaagaaggcccctgcaagatgccctcccctcagtattggacttcacagcctccaggaccataagccaataaatttttgttcattataaatttcccagtctgtggtattctgttatagcaacactcaatttatgcattacttccagattcttatggctatacctacttctcacagtttgtattcacccctccttcaaccaagtacccttaacacagttcccatagtcacaaagccaggtcactgaagctgccctctctccaaccacacacatatagatcaaatgaccccagacatagagctgattgagaaggagggaccagtacgagctctgcttccccagcagcttcctggaaagaagaggcaatacaacccaacccaaaagtgcaagagaagtaacacctcatgggatgagcttaattaatcaatgggagaggacactagaagacactagaggatctcccttcctccctttctttcccacttcaccccctccagtctctgaaccatgagctatttcaaaggtgcagtaatgctatatttggcttctctgaagatatcctatgaggccaagtcatcagctttgttcattatctaagagtggtggccagctcaccagcacttcccatcatgtttgccctccctctttcccttgtgttacttcccattttcccttacttctgctttcttggcattaaattctactctgcaatgttaggatataagtttttgcctcagattctgttttctaggaaacccatgctaagacaacactggcagtggccctggaaaagtaaacctcatgatggatttggagttggattgttcactgatctgaaggacagaggactccacttaagtggtaagcagtgtagctatgaactctgccacgcaggcctcacaattactgaggcttcttttacctgtggttaactgggacacagaacagcaggaaattgagtgtagaggttatcaagtagctgcttcacttaattggtataattttatggagttaacctggtttagagtccagagaacattccacatagcctagaaagggtagttatttgtccttaccataatcaagtcatactttgaatatgagttttccttccctgttcagcaccacttctcttagacttaagaatgcctgatctgttgatattatgtcccatgtaacattgcctgagacaaagatatccatgtaccttaaa

SEQ ID NO: 19 - protein, 140 aa, homo sapiens
MGFQKFSPFLALSILVLLQAGSLHAAPFRSALESSPADPATLSEDEARLLLAALVQDYVQMKASELEQEQEREGSSLDSPRSKRCGNLSTCMLGTYTQDFNKFHTFPQTAIGVGAPGKKRDMSSDLERDHRPHVSMPQNA

SEQ ID NO: 20 - protein, 128 aa, homo sapiens
MGFQKFSPFLALSILVLLQAGSLHAAPFRSALESSPADPATLSEDEARLLLAALVQDYVQMKASELEQEQEREGSRIIAQKRACDTATCVTHRLAGLLSRSGGVVKNNFVPTNVGSKAFGRRRRDLQA

SEQ ID NO: 21 - protein, 141 aa, homo sapiens
MGFQKFSPFLALSILVLLQAGSLHAAPFRSALESSPADPATLSEDEARLLLAALVQDYVQMKASELEQEQEREGSSLDSPRSKRCGNLSTCMLGTYTQDFNKFHTFPQTAIGVGAPGKKRDMSSDLERDHRPHVSMPQNAN

SEQ ID NO: 22 - protein, 116 aa, homo sapiens
APFRSALESSPADPATLSEDEARLLLAALVQDYVQMKASELEQEQEREGSSLDSPRSKRCGNLSTCMLGTYTQDFNKFHTFPQTAIGVGAPGKKRDMSSDLERDHRPHVSMPQNAN

SEQ ID NO: 23 - protein, 212 aa, homo sapiens
MNSFSTSAFGPVAFSLGLLLVLPAAFPAPVPPGEDSKDVAAPHRQPLTSSERIDKQIRYILDGISALRKETCNKSNMCESSKEALAENNLNLPKMAEKDGCFQSGFNEETCLVKIITGLLEFEVYLEYLQNRFESSEEQARAVQMSTKVLIQFLQKKAKNLDAITTPDPTTNASLLTKLQAQNQWLQDMTTHLILRSFKEFLQSSLRALRQM

SEQ ID NO: 24 - protein, 136 aa, homo sapiens
MCESSKEALAENNLNLPKMAEKDGCFQSGFNEETCLVKIITGLLEFEVYLEYLQNRFESSEEQARAVQMSTKVLIQFLQKKAKNLDAITTPDPTTNASLLTKLQAQNQWLQDMTTHLILRSFKEFLQSSLRALRQM